European Patent Specification EP 3 470 430 B1, published August 28, 2024. Title: ANTIBODY FOR BINDING TO INTERLEUKIN 4 RECEPTOR. Applicant: SUZHOU CONNECT BIOPHARMACEUTICALS LTD. The sequence listing filed with the application follows.

SEQUENCE LISTING (94 sequences)

SEQ ID NO: 1 - protein, 12 aa, Artificial sequence
  LCDR1-1
RASQSVSNSYLA

SEQ ID NO: 2 - protein, 12 aa, Artificial sequence
  LCDR1-2
RASQSVSSSYLA

SEQ ID NO: 3 - protein, 7 aa, Artificial sequence
  LCDR2-1
GASSRAT

SEQ ID NO: 4 - protein, 7 aa, Artificial sequence
  LCDR2-2
GASSRAP

SEQ ID NO: 5 - protein, 10 aa, Artificial sequence
  LCDR3-1
QQYGSSPPWT

SEQ ID NO: 6 - protein, 10 aa, Artificial sequence
  LCDR3-2
QQYDHSPPWT

SEQ ID NO: 7 - protein, 10 aa, Artificial sequence
  LCDR3-3
QQYGSSAGWT

SEQ ID NO: 8 - protein, 10 aa, Artificial sequence
  LCDR3-4
QQYDHSAGWT

SEQ ID NO: 9 - protein, 23 aa, Artificial sequence
  LFR1-1
EIVLTQSPGTLSLSPGERATLSC

SEQ ID NO: 10 - protein, 15 aa, Artificial sequence
  LFR2-1
WYQQKPGQAPRLLIF

SEQ ID NO: 11 - protein, 15 aa, Artificial sequence
  LFR2-2
WYQQKPGQAPRLLIY

SEQ ID NO: 12 - protein, 32 aa, Artificial sequence
  LFR3-1
GIPDRFSGSGSGTDFTLTISRLEPEDFAVYYC

SEQ ID NO: 13 - protein, 10 aa, Artificial sequence
  LFR4-1
FGQGTKVEIK

SEQ ID NO: 14 - protein, 5 aa, Artificial sequence
  HCDR1-1
RNAMF

SEQ ID NO: 15 - protein, 5 aa, Artificial sequence
  HCDR1-2
RNAMH

SEQ ID NO: 16 - protein, 5 aa, Artificial sequence
  HCDR1-3
DYAMF

SEQ ID NO: 17 - protein, 17 aa, Artificial sequence
  HCDR2-1
GIGTGGATNYADSVKGR

SEQ ID NO: 18 - protein, 17 aa, Artificial sequence
  HCDR2-2
GIGTGGATSYADSVKGR

SEQ ID NO: 19 - protein, 7 aa, Artificial sequence
  HCDR3-1
GRYYFDY

SEQ ID NO: 20 - protein, 7 aa, Artificial sequence
  HCDR3-2
GRYYFPW

SEQ ID NO: 21 - protein, 30 aa, Artificial sequence
  HFR1-1
EVQLVESGGGLVHPGGSLRLSCAGSGFTFS

SEQ ID NO: 22 - protein, 30 aa, Artificial sequence
  HFR1-2
EVQLVQSGGGLVQPGGSLRLSCAGSGFTFS

SEQ ID NO: 23 - protein, 30 aa, Artificial sequence
  HFR1-3
EVQLVQSGGGLVHPGGSLRLSCAASGFTFS

SEQ ID NO: 24 - protein, 30 aa, Artificial sequence
  HFR1-4
EVQLVQSGGGLVHPGGSLRLSCAGSGFTFS

SEQ ID NO: 25 - protein, 30 aa, Artificial sequence
  HFR1-5
EVQLVESGGGLVQPGGSLRLSCAGSGFTFS

SEQ ID NO: 26 - protein, 30 aa, Artificial sequence
  HFR1-6
EVQLVESGGGLVHPGGSLRLSCAASGFTFS

SEQ ID NO: 27 - protein, 30 aa, Artificial sequence
  HFR1-7
EVQLVQSGGGLVQPGGSLRLSCAASGFTFS

SEQ ID NO: 28 - protein, 30 aa, Artificial sequence
  HFR1-8
EVQLVESGGGLVQPGGSLRLSCAASGFTFS

SEQ ID NO: 29 - protein, 30 aa, Artificial sequence
  HFR1-9
EVQLVQSGGGLVHPGRSLRLSCAGSGFTFS

SEQ ID NO: 30 - protein, 30 aa, Artificial sequence
  HFR1-10
EVQLVQSGGGLVHPGGSLRLTCAGSGFTFS

SEQ ID NO: 31 - protein, 30 aa, Artificial sequence
  HFR1-11
EVQLVQSGGGLVHPGGSLRLSCAGSGFTFD

SEQ ID NO: 32 - protein, 14 aa, Artificial sequence
  HFR2-1
WVRQAPGKGLEWVS

SEQ ID NO: 33 - protein, 14 aa, Artificial sequence
  HFR2-2
WVRQAPGEGLEWVS

SEQ ID NO: 34 - protein, 31 aa, Artificial sequence
  HFR3-1
FTISRDNAKNSLYLQMNSLRAEDMAVYYCAR

SEQ ID NO: 35 - protein, 31 aa, Artificial sequence
  HFR3-2
FTISRDNAKNSLYLQMNSLRAEDTAVYYCAR

SEQ ID NO: 36 - protein, 31 aa, Artificial sequence
  HFR3-3
FTISRDEAKNSLYLQMNSLRAEDMAVYYCAR

SEQ ID NO: 37 - protein, 31 aa, Artificial sequence
  HFR3-4
FTISRDNAKNSLYLQMNSLRAGDMAVYYCAR

SEQ ID NO: 38 - protein, 11 aa, Artificial sequence
  HFR4-1
WGQGTLVTVSS

SEQ ID NO: 39 - protein, 109 aa, Artificial sequence
  VL（L1007）
EIVLTQSPGTLSLSPGERATLSCRASQSVSNSYLAWYQQKPGQAPRLLIFGASSRATGIPDRFSGSGSGTDFTLTISRLEPEDFAVYYCQQYGSSPPWTFGQGTKVEIK

SEQ ID NO: 40 - protein, 109 aa, Artificial sequence
  VL（L1008）
EIVLTQSPGTLSLSPGERATLSCRASQSVSSSYLAWYQQKPGQAPRLLIYGASSRATGIPDRFSGSGSGTDFTLTISRLEPEDFAVYYCQQYGSSPPWTFGQGTKVEIK

SEQ ID NO: 41 - protein, 109 aa, Artificial sequence
  VL（L1009）
EIVLTQSPGTLSLSPGERATLSCRASQSVSSSYLAWYQQKPGQAPRLLIFGASSRAPGIPDRFSGSGSGTDFTLTISRLEPEDFAVYYCQQYGSSPPWTFGQGTKVEIK

SEQ ID NO: 42 - protein, 109 aa, Artificial sequence
  VL（L1010）
EIVLTQSPGTLSLSPGERATLSCRASQSVSNSYLAWYQQKPGQAPRLLIYGASSRATGIPDRFSGSGSGTDFTLTISRLEPEDFAVYYCQQYGSSPPWTFGQGTKVEIK

SEQ ID NO: 43 - protein, 109 aa, Artificial sequence
  VL（L1011）
EIVLTQSPGTLSLSPGERATLSCRASQSVSNSYLAWYQQKPGQAPRLLIFGASSRAPGIPDRFSGSGSGTDFTLTISRLEPEDFAVYYCQQYGSSPPWTFGQGTKVEIK

SEQ ID NO: 44 - protein, 109 aa, Artificial sequence
  VL（L1012）
EIVLTQSPGTLSLSPGERATLSCRASQSVSSSYLAWYQQKPGQAPRLLIYGASSRAPGIPDRFSGSGSGTDFTLTISRLEPEDFAVYYCQQYGSSPPWTFGQGTKVEIK

SEQ ID NO: 45 - protein, 109 aa, Artificial sequence
  VL（L1016）
EIVLTQSPGTLSLSPGERATLSCRASQSVSSSYLAWYQQKPGQAPRLLIFGASSRATGIPDRFSGSGSGTDFTLTISRLEPEDFAVYYCQQYDHSPPWTFGQGTKVEIK

SEQ ID NO: 46 - protein, 109 aa, Artificial sequence
  VL（L1017）
EIVLTQSPGTLSLSPGERATLSCRASQSVSSSYLAWYQQKPGQAPRLLIFGASSRATGIPDRFSGSGSGTDFTLTISRLEPEDFAVYYCQQYGSSAGWTFGQGTKVEIK

SEQ ID NO: 47 - protein, 109 aa, Artificial sequence
  VL（L1018）
EIVLTQSPGTLSLSPGERATLSCRASQSVSSSYLAWYQQKPGQAPRLLIFGASSRATGIPDRFSGSGSGTDFTLTISRLEPEDFAVYYCQQYDHSAGWTFGQGTKVEIK

SEQ ID NO: 48 - protein, 109 aa, Artificial sequence
  VL（L1013）
EIVLTQSPGTLSLSPGERATLSCRASQSVSNSYLAWYQQKPGQAPRLLIFGASSRATGIPDRFSGSGSGTDFTLTISRLEPEDFAVYYCQQYDHSPPWTFGQGTKVEIK

SEQ ID NO: 49 - protein, 109 aa, Artificial sequence
  VL（L1014）
EIVLTQSPGTLSLSPGERATLSCRASQSVSSSYLAWYQQKPGQAPRLLIYGASSRATGIPDRFSGSGSGTDFTLTISRLEPEDFAVYYCQQYDHSPPWTFGQGTKVEIK

SEQ ID NO: 50 - protein, 109 aa, Artificial sequence
  VL（L1015）
EIVLTQSPGTLSLSPGERATLSCRASQSVSSSYLAWYQQKPGQAPRLLIFGASSRAPGIPDRFSGSGSGTDFTLTISRLEPEDFAVYYCQQYDHSPPWTFGQGTKVEIK

SEQ ID NO: 51 - protein, 109 aa, Artificial sequence
  VL（L1023）
EIVLTQSPGTLSLSPGERATLSCRASQSVSSSYLAWYQQKPGQAPRLLIYGASSRAPGIPDRFSGSGSGTDFTLTISRLEPEDFAVYYCQQYDHSAGWTFGQGTKVEIK

SEQ ID NO: 52 - protein, 109 aa, Artificial sequence
  VL（L1024）
EIVLTQSPGTLSLSPGERATLSCRASQSVSNSYLAWYQQKPGQAPRLLIFGASSRAPGIPDRFSGSGSGTDFTLTISRLEPEDFAVYYCQQYDHSAGWTFGQGTKVEIK

SEQ ID NO: 53 - protein, 109 aa, Artificial sequence
  VL（L1022）
EIVLTQSPGTLSLSPGERATLSCRASQSVSNSYLAWYQQKPGQAPRLLIYGASSRATGIPDRFSGSGSGTDFTLTISRLEPEDFAVYYCQQYDHSAGWTFGQGTKVEIK

SEQ ID NO: 54 - protein, 109 aa, Artificial sequence
  VL（L1021）
EIVLTQSPGTLSLSPGERATLSCRASQSVSSSYLAWYQQKPGQAPRLLIFGASSRAPGIPDRFSGSGSGTDFTLTISRLEPEDFAVYYCQQYDHSAGWTFGQGTKVEIK

SEQ ID NO: 55 - protein, 109 aa, Artificial sequence
  VL（L1020）
EIVLTQSPGTLSLSPGERATLSCRASQSVSSSYLAWYQQKPGQAPRLLIYGASSRATGIPDRFSGSGSGTDFTLTISRLEPEDFAVYYCQQYDHSAGWTFGQGTKVEIK

SEQ ID NO: 56 - protein, 109 aa, Artificial sequence
  VL（L1019）
EIVLTQSPGTLSLSPGERATLSCRASQSVSNSYLAWYQQKPGQAPRLLIFGASSRATGIPDRFSGSGSGTDFTLTISRLEPEDFAVYYCQQYDHSAGWTFGQGTKVEIK

SEQ ID NO: 57 - protein, 109 aa, Artificial sequence
  VL（L1000）
EIVLTQSPGTLSLSPGERATLSCRASQSVSSSYLAWYQQKPGQAPRLLIFGASSRATGIPDRFSGSGSGTDFTLTISRLEPEDFAVYYCQQYGSSPPWTFGQGTKVEIK

SEQ ID NO: 58 - protein, 109 aa, Artificial sequence
  VL（L1001）
EIVLTQSPGTLSLSPGERATLSCRASQSVSNSYLAWYQQKPGQAPRLLIYGASSRAPGIPDRFSGSGSGTDFTLTISRLEPEDFAVYYCQQYDHSAGWTFGQGTKVEIK

SEQ ID NO: 59 - protein, 115 aa, Artificial sequence
  VH（H1009）
EVQLVESGGGLVHPGGSLRLSCAGSGFTFSRNAMFWVRQAPGKGLEWVSGIGTGGATNYADSVKGRFTISRDNAKNSLYLQMNSLRAEDMAVYYCARGRYYFDYWGQGTLVTVSS

SEQ ID NO: 60 - protein, 115 aa, Artificial sequence
  VH（H1010）
EVQLVQSGGGLVQPGGSLRLSCAGSGFTFSRNAMFWVRQAPGKGLEWVSGIGTGGATNYADSVKGRFTISRDNAKNSLYLQMNSLRAEDMAVYYCARGRYYFDYWGQGTLVTVSS

SEQ ID NO: 61 - protein, 115 aa, Artificial sequence
  VH（H1011）
EVQLVQSGGGLVHPGGSLRLSCAASGFTFSRNAMFWVRQAPGKGLEWVSGIGTGGATNYADSVKGRFTISRDNAKNSLYLQMNSLRAEDMAVYYCARGRYYFDYWGQGTLVTVSS

SEQ ID NO: 62 - protein, 115 aa, Artificial sequence
  VH（H1007）
EVQLVQSGGGLVHPGGSLRLSCAGSGFTFSRNAMFWVRQAPGKGLEWVSGIGTGGATSYADSVKGRFTISRDNAKNSLYLQMNSLRAEDMAVYYCARGRYYFDYWGQGTLVTVSS

SEQ ID NO: 63 - protein, 115 aa, Artificial sequence
  VH（H1008）
EVQLVQSGGGLVHPGGSLRLSCAGSGFTFSRNAMFWVRQAPGKGLEWVSGIGTGGATNYADSVKGRFTISRDNAKNSLYLQMNSLRAEDTAVYYCARGRYYFDYWGQGTLVTVSS

SEQ ID NO: 64 - protein, 115 aa, Artificial sequence
  VH（H1015）
EVQLVESGGGLVQPGGSLRLSCAGSGFTFSRNAMFWVRQAPGKGLEWVSGIGTGGATNYADSVKGRFTISRDNAKNSLYLQMNSLRAEDMAVYYCARGRYYFDYWGQGTLVTVSS

SEQ ID NO: 65 - protein, 115 aa, Artificial sequence
  VH（H1013）
EVQLVESGGGLVHPGGSLRLSCAASGFTFSRNAMFWVRQAPGKGLEWVSGIGTGGATNYADSVKGRFTISRDNAKNSLYLQMNSLRAEDMAVYYCARGRYYFDYWGQGTLVTVSS

SEQ ID NO: 66 - protein, 115 aa, Artificial sequence
  VH（H1014）
EVQLVQSGGGLVQPGGSLRLSCAASGFTFSRNAMFWVRQAPGKGLEWVSGIGTGGATNYADSVKGRFTISRDNAKNSLYLQMNSLRAEDMAVYYCARGRYYFDYWGQGTLVTVSS

SEQ ID NO: 67 - protein, 115 aa, Artificial sequence
  VH（H1012）
EVQLVQSGGGLVHPGGSLRLSCAGSGFTFSRNAMFWVRQAPGKGLEWVSGIGTGGATSYADSVKGRFTISRDNAKNSLYLQMNSLRAEDTAVYYCARGRYYFDYWGQGTLVTVSS

SEQ ID NO: 68 - protein, 115 aa, Artificial sequence
  VH（H1016）
EVQLVQSGGGLVHPGGSLRLSCAGSGFTFSRNAMFWVRQAPGKGLEWVSGIGTGGATNYADSVKGRFTISRDNAKNSLYLQMNSLRAEDMAVYYCARGRYYFPWWGQGTLVTVSS

SEQ ID NO: 69 - protein, 115 aa, Artificial sequence
  VH（H1017）
EVQLVESGGGLVHPGGSLRLSCAGSGFTFSRNAMFWVRQAPGKGLEWVSGIGTGGATNYADSVKGRFTISRDNAKNSLYLQMNSLRAEDMAVYYCARGRYYFPWWGQGTLVTVSS

SEQ ID NO: 70 - protein, 115 aa, Artificial sequence
  VH（H1018）
EVQLVQSGGGLVQPGGSLRLSCAGSGFTFSRNAMFWVRQAPGKGLEWVSGIGTGGATNYADSVKGRFTISRDNAKNSLYLQMNSLRAEDMAVYYCARGRYYFPWWGQGTLVTVSS

SEQ ID NO: 71 - protein, 115 aa, Artificial sequence
  VH（H1019）
EVQLVQSGGGLVHPGGSLRLSCAASGFTFSRNAMFWVRQAPGKGLEWVSGIGTGGATNYADSVKGRFTISRDNAKNSLYLQMNSLRAEDMAVYYCARGRYYFPWWGQGTLVTVSS

SEQ ID NO: 72 - protein, 115 aa, Artificial sequence
  VH（H1020）
EVQLVQSGGGLVHPGGSLRLSCAGSGFTFSRNAMFWVRQAPGKGLEWVSGIGTGGATSYADSVKGRFTISRDNAKNSLYLQMNSLRAEDMAVYYCARGRYYFPWWGQGTLVTVSS

SEQ ID NO: 73 - protein, 115 aa, Artificial sequence
  VH（H1021）
EVQLVQSGGGLVHPGGSLRLSCAGSGFTFSRNAMFWVRQAPGKGLEWVSGIGTGGATNYADSVKGRFTISRDNAKNSLYLQMNSLRAEDTAVYYCARGRYYFPWWGQGTLVTVSS

SEQ ID NO: 74 - protein, 115 aa, Artificial sequence
  VH（H1033）
EVQLVQSGGGLVHPGRSLRLSCAGSGFTFSRNAMFWVRQAPGKGLEWVSGIGTGGATNYADSVKGRFTISRDNAKNSLYLQMNSLRAEDMAVYYCARGRYYFDYWGQGTLVTVSS

SEQ ID NO: 75 - protein, 115 aa, Artificial sequence
  VH（H1034）
EVQLVQSGGGLVHPGGSLRLTCAGSGFTFSRNAMFWVRQAPGKGLEWVSGIGTGGATNYADSVKGRFTISRDNAKNSLYLQMNSLRAEDMAVYYCARGRYYFDYWGQGTLVTVSS

SEQ ID NO: 76 - protein, 115 aa, Artificial sequence
  VH（H1035）
EVQLVQSGGGLVHPGGSLRLSCAGSGFTFSRNAMHWVRQAPGKGLEWVSGIGTGGATNYADSVKGRFTISRDNAKNSLYLQMNSLRAEDMAVYYCARGRYYFDYWGQGTLVTVSS

SEQ ID NO: 77 - protein, 115 aa, Artificial sequence
  VH（H1036）
EVQLVQSGGGLVHPGGSLRLSCAGSGFTFSRNAMFWVRQAPGEGLEWVSGIGTGGATNYADSVKGRFTISRDNAKNSLYLQMNSLRAEDMAVYYCARGRYYFDYWGQGTLVTVSS

SEQ ID NO: 78 - protein, 115 aa, Artificial sequence
  VH（H1037）
EVQLVQSGGGLVHPGGSLRLSCAGSGFTFSRNAMFWVRQAPGKGLEWVSGIGTGGATNYADSVKGRFTISRDEAKNSLYLQMNSLRAEDMAVYYCARGRYYFDYWGQGTLVTVSS

SEQ ID NO: 79 - protein, 115 aa, Artificial sequence
  VH（H1039）
EVQLVQSGGGLVHPGGSLRLSCAGSGFTFSRNAMFWVRQAPGKGLEWVSGIGTGGATNYADSVKGRFTISRDNAKNSLYLQMNSLRAGDMAVYYCARGRYYFDYWGQGTLVTVSS

SEQ ID NO: 80 - protein, 115 aa, Artificial sequence
  VH（H1038）
EVQLVQSGGGLVHPGGSLRLSCAGSGFTFDDYAMFWVRQAPGKGLEWVSGIGTGGATNYADSVKGRFTISRDNAKNSLYLQMNSLRAEDMAVYYCARGRYYFDYWGQGTLVTVSS

SEQ ID NO: 81 - protein, 115 aa, Artificial sequence
  VH（H1028）
EVQLVQSGGGLVQPGGSLRLSCAASGFTFSRNAMFWVRQAPGKGLEWVSGIGTGGATSYADSVKGRFTISRDNAKNSLYLQMNSLRAEDTAVYYCARGRYYFPWWGQGTLVTVSS

SEQ ID NO: 82 - protein, 115 aa, Artificial sequence
  VH（H1027）
EVQLVESGGGLVHPGGSLRLSCAASGFTFSRNAMFWVRQAPGKGLEWVSGIGTGGATSYADSVKGRFTISRDNAKNSLYLQMNSLRAEDTAVYYCARGRYYFPWWGQGTLVTVSS

SEQ ID NO: 83 - protein, 115 aa, Artificial sequence
  VH（H1026）
EVQLVESGGGLVQPGGSLRLSCAGSGFTFSRNAMFWVRQAPGKGLEWVSGIGTGGATSYADSVKGRFTISRDNAKNSLYLQMNSLRAEDTAVYYCARGRYYFPWWGQGTLVTVSS

SEQ ID NO: 84 - protein, 115 aa, Artificial sequence
  VH（H1030）
EVQLVESGGGLVQPGGSLRLSCAASGFTFSRNAMFWVRQAPGKGLEWVSGIGTGGATNYADSVKGRFTISRDNAKNSLYLQMNSLRAEDTAVYYCARGRYYFPWWGQGTLVTVSS

SEQ ID NO: 85 - protein, 115 aa, Artificial sequence
  VH（H1029）
EVQLVESGGGLVQPGGSLRLSCAASGFTFSRNAMFWVRQAPGKGLEWVSGIGTGGATSYADSVKGRFTISRDNAKNSLYLQMNSLRAEDMAVYYCARGRYYFPWWGQGTLVTVSS

SEQ ID NO: 86 - protein, 115 aa, Artificial sequence
  VH（H1025）
EVQLVQSGGGLVHPGGSLRLSCAASGFTFSRNAMFWVRQAPGKGLEWVSGIGTGGATSYADSVKGRFTISRDNAKNSLYLQMNSLRAEDTAVYYCARGRYYFPWWGQGTLVTVSS

SEQ ID NO: 87 - protein, 115 aa, Artificial sequence
  VH（H1024）
EVQLVQSGGGLVQPGGSLRLSCAGSGFTFSRNAMFWVRQAPGKGLEWVSGIGTGGATSYADSVKGRFTISRDNAKNSLYLQMNSLRAEDTAVYYCARGRYYFPWWGQGTLVTVSS

SEQ ID NO: 88 - protein, 115 aa, Artificial sequence
  VH（H1023）
EVQLVESGGGLVHPGGSLRLSCAGSGFTFSRNAMFWVRQAPGKGLEWVSGIGTGGATSYADSVKGRFTISRDNAKNSLYLQMNSLRAEDTAVYYCARGRYYFPWWGQGTLVTVSS

SEQ ID NO: 89 - protein, 115 aa, Artificial sequence
  VH（H1022）
EVQLVQSGGGLVHPGGSLRLSCAGSGFTFSRNAMFWVRQAPGKGLEWVSGIGTGGATSYADSVKGRFTISRDNAKNSLYLQMNSLRAEDTAVYYCARGRYYFPWWGQGTLVTVSS

SEQ ID NO: 90 - protein, 115 aa, Artificial sequence
  VH（H1032）
EVQLVESGGGLVQPGGSLRLSCAASGFTFSRNAMFWVRQAPGKGLEWVSGIGTGGATNYADSVKGRFTISRDNAKNSLYLQMNSLRAEDMAVYYCARGRYYFPWWGQGTLVTVSS

SEQ ID NO: 91 - protein, 115 aa, Artificial sequence
  VH（H1031）
EVQLVESGGGLVQPGGSLRLSCAASGFTFSRNAMFWVRQAPGKGLEWVSGIGTGGATSYADSVKGRFTISRDNAKNSLYLQMNSLRAEDTAVYYCARGRYYFDYWGQGTLVTVSS

SEQ ID NO: 92 - protein, 115 aa, Artificial sequence
  VH（H1000）
EVQLVQSGGGLVHPGGSLRLSCAGSGFTFSRNAMFWVRQAPGKGLEWVSGIGTGGATNYADSVKGRFTISRDNAKNSLYLQMNSLRAEDMAVYYCARGRYYFDYWGQGTLVTVSS

SEQ ID NO: 93 - protein, 115 aa, Artificial sequence
  VH（H1001）
EVQLVESGGGLVQPGGSLRLSCAASGFTFSRNAMFWVRQAPGKGLEWVSGIGTGGATSYADSVKGRFTISRDNAKNSLYLQMNSLRAEDTAVYYCARGRYYFPWWGQGTLVTVSS

SEQ ID NO: 94 - protein, 209 aa, human
  sIL4Rα
GNMKVLQEPTCVSDYMSISTCEWKMNGPTNCSTELRLLYQLVFLLSEAHTCIPENNGGAGCVCHLLMDDVVSADNYTLDLWAGQQLLWKGSFKPSEHVKPRAPGNLTVHTNVSDTLLLTWSNPYPPDNYLYNHLTYAVNIWSENDPADFRIYNVTYLEPSLRIAASTLKSGISYRARVRAWAQCYNTTWSEWSPSTKWHNSYREPFEQH